European Patent Application EP 4 545 091 A1, published April 30, 2025. Title: Transmembrane Serine Protease and Neutrophil Elastase Inhibitors. Applicant: Universität Ulm. The sequence listing filed with the application follows.

SEQUENCE LISTING (2 sequences)

SEQ ID NO: 1 - protein, 51 aa, Homo sapiens
CNLPIVRGPCRAFIQLWAFDAVKGKCVLFPYGGCQGNGNKFYSEKECREYC

SEQ ID NO: 2 - protein, 61 aa, Homo sapiens
VAACNLPIVRGPCRAFIQLWAFDAVKGKCVLFPYGGCQGNGNKFYSEKECREYCGVPGDGD